European Patent Specification EP 4 055 189 B1, published January 1, 2025. Title: BIVALENT REVERSE PRIMER. Applicant: Mirnax Biosens, S.L. Application EP20382336.4. The sequence listing filed with the application follows.

SEQUENCE LISTING (31 sequences)

SEQ ID NO: 1 - DNA, 25 bp, Artificial Sequence
  miR-127-3p-F
aatactacattaatgtcattcggat

SEQ ID NO: 2 - RNA, 22 nt, Artificial Sequence
  miR-127-3p-M
ucggauccgucugagcuuggcu

SEQ ID NO: 3 - DNA, 14 bp, Artificial Sequence
  miR-127-3p-P
atccgtctgagctt

SEQ ID NO: 4 - DNA, 25 bp, Artificial Sequence
  miR-127-3p-R
aaccgatactgtaattacatcataa

SEQ ID NO: 5 - DNA, 25 bp, Artificial Sequence
  miR-144-5p-F
aatactacattaatgtcatggatat

SEQ ID NO: 6 - RNA, 22 nt, Artificial Sequence
  miR-144-5p-M
ggauaucaucauauacuguaag

SEQ ID NO: 7 - DNA, 14 bp, Artificial Sequence
  miR-144-5p-P
atcatcatatactg

SEQ ID NO: 8 - DNA, 25 bp, Artificial Sequence
  miR-144-5p-R
acattctactgtaattacatcataa

SEQ ID NO: 9 - DNA, 25 bp, Artificial Sequence
  miR-185-5p-F
aatactacattaatgtcattggaga

SEQ ID NO: 10 - RNA, 22 nt, Artificial Sequence
  miR-185-5p-M
uggagagaaaggcaguuccuga

SEQ ID NO: 11 - DNA, 14 bp, Artificial Sequence
  miR-185-5p-P
gagaaaggcagttc

SEQ ID NO: 12 - DNA, 25 bp, Artificial Sequence
  miR-185-5p-R
aggacttactgtaattacatcataa

SEQ ID NO: 13 - DNA, 24 bp, Artificial Sequence
  miR-1246-F
aatactacattaatgtcataatgg

SEQ ID NO: 14 - RNA, 19 nt, Artificial Sequence
  miR-1246-M
aauggauuuuuggagcagg

SEQ ID NO: 15 - DNA, 15 bp, Artificial Sequence
  miR-1246-P
tggatttttggagca

SEQ ID NO: 16 - DNA, 24 bp, Artificial Sequence
  miR-1246-R
cgtcctactgtaattacatcataa

SEQ ID NO: 17 - DNA, 28 bp, Artificial Sequence
  uSEQ RTqPCR MiRNAX1 Forward
ctgctggcacgkagttagccaaaaaaaa

SEQ ID NO: 18 - DNA, 23 bp, Artificial Sequence
  uSEQ RTqPCR MiRNAX1 Reverse
acacggyccagactctttttttt

SEQ ID NO: 19 - DNA, 26 bp, Artificial Sequence
  uSEQ RTqPCR MiRNAX2 Forward
gacarccatgcascacctaaaaaaaa

SEQ ID NO: 20 - DNA, 20 bp, Artificial Sequence
  uSEQ RTqPCR MiRNAX2 Reverse
gcaacgcgaagatttttttt

SEQ ID NO: 21 - DNA, 23 bp, Artificial Sequence
  uSEQ RTqPCR MiRNAX3 Forward
ctcacccgtcgccrcaaaaaaaa

SEQ ID NO: 22 - DNA, 25 bp, Artificial Sequence
  uSEQ RTqPCR MiRNAX3 Reverse
gaagagtttgatcatggtttttttt

SEQ ID NO: 23 - DNA, 2308 bp, Staphylococcus aureus
  subsp. aureus ATCC 12600
caccccaatcatttgtcccaccttcgacggctagctcctaaaaggttactccaccggcttcgggtgttacaaactctcgtggtgtgacgggcggtgtgtacaagacccgggaacgtattcaccgtagcatgctgatctacgattactagcgattccagcttcatgtagtcgagttgcagactacaatccgaactgagaacaactttatgggatttgcttgacctcgcggtttcgctgccctttgtattgtccattgtagcacgtgtgtagcccaaatcataaggggcatgatgatttgacgtcatccccaccttcctccggtttgtcaccggcagtcaacttagagtgcccaacttaatgatggcaactaagcttaagggttgcgctcgttgcgggacttaacccaacatctcacgacacgagctgacgacaaccatgcaccacctgtcactttgtcccccgaaggggaaggctctatctctagagttgtcaaaggatgtcaagatttggtaaggttcttcgcgttgcttcgaattaaaccacatgctccaccgcttgtgcgggtccccgtcaattcctttgagtttcaaccttgcggtcgtactccccaggcggagtgcttaatgcgttagctgcagcactaaggggcggaaaccccctaacacttagcactcatcgtttacggcgtggactaccagggtatctaatcctgtttgatccccacgctttcgcacatcagcgtcagttacagaccagaaagtcgccttcgccactggtgttcctccatatctctgcgcatttcaccgctacacatggaattccactttcctctcaccccaatcatttgtcccaccttcgacggctagctcctaaaaggttactccaccggcttcgggtgttacaaactctcgtggtgtgacgggcggtgtgtacaagacccgggaacgtattcaccgtagcatgctgatctacgattactagcgattccagcttcatgtagtcgagttgcagactacaatccgaactgagaacaactttatgggatttgcttgacctcgcggtttcgctgccctttgtattgtccattgtagcacgtgtgtagcccaaatcataaggggcatgatgatttgacgtcatccccaccttcctccggtttgtcaccggcagtcaacttagagtgcccaacttaatgatggcaactaagcttaagggttgcgctcgttgcgggacttaacccaacatctcacgacacgagctgacgacaaccatgcaccacctgtcactttgtcccccgaaggggaaggctctatctctagagttgtcaaaggatgtcaagatttggtaaggttcttcgcgttgcttcgaattaaaccacatgctccaccgcttgtgcgggtccccgtcaattcctttgagtttcaaccttgcggtcgtactccccaggcggagtgcttaatgcgttagctgcagcactaaggggcggaaaccccctaacacttagcactcatcgtttacggcgtggactaccagggtatctaatcctgtttgatccccacgctttcgcacatcagcgtcagttacagaccagaaagtcgccttcgccactggtgttcctccatatctctgcgcatttcaccgctacacatggaattccactttcctcttctgcactcaagttttccagtttccaatgaccctccacggttgagccgtgggctttcacatcagacttaaaaaaccgcctacgcgcgctttacgcccaataattccggataacgcttgccacctacgtattaccgcggctgctggcacgtagttagccgtggctttctgattaggtaccgtcaagatgtgcacagttacttacacatatgttcttccctaataacagagttttacgatccgaagaccttcatcactcacgcggcgttgctccgtcaggctttcgcccattgcggaagattccctactgctgcctcccgtaggagtctggaccgtgtctcagttccagtgtggccgatcaccctctcaggtcggctatgcatcgttgccttggtaagccgttaccttaccaactagctaatgcagcgcggatccatctataagtgacagcaagaccgtctttcacttttgaaccatgcggttcaaaatattatccggtattagctccggtttcccgaagttatcccagtcttataggtaggttatccacgtgttactcacccgtccgccgctaacatcagagaagcaagcttctcgtccgttcgctcgacttgcatgtattaggcacgccgccagcgttcatcct

SEQ ID NO: 24 - DNA, 1450 bp, Escherichia coli
  ATCC 117757
  misc_feature 598,599,1059: /note="n= a or g or c or t/u"
cgccctcccgaagttaagctacctacttcttttgcaacccactcccatggtgtgacgggcggtgtgtacaaggcccgggaacgtattcaccgtggcattctgatccacgattactagcgattccgacttcatggagtcgagttgcagactccaatccggactacgacgcactttatgaggtccgcttgctctcgcgaggtcgcttctctttgtatgcgccattgtagcacgtgtgtagccctggtcgtaagggccatgatgacttgacgtcatccccaccttcctccagtttatcactggcagtctcctttgagttcccggccggaccgctggcaacaaaggataagggttgcgctcgttgcgggacttaacccaacatttcacaacacgagctgacgacagccatgcagcacctgtctcacggttcccgaaggcacattctcatctctgaaaacttccgtggatgtcaagaccaggtaaggttcttcgcgttgcatcgaattaaaccacatgctccaccgcttgtgcggcccccgtcaattcatttgagttttaaccttgcggccgtactccccaggcggtcgacttaacgcgttanntccggaagccacgcctcaagggcacaacctccaagtcgacatcgtttacggcgtggactaccagggtatctaatcctgtttgctccccacgctttcgcacctgagcgtcagtcttcgtccagggggccgccttcgccaccggtattcctccagatctctacgcatttcaccgctacacctggaattctacccccctctacgagactcaagcttgccagtatcagatgcagttcccaggttgagcccggggatttcacatctgacttaacaaaccgcctgcgtgcgctttacgcccagtaattccgattaacgcttgcaccctccgtattaccgcggctgctggcacggagttagccggtgcttcttctgcgggtaacgtcaatgagcaaaggtattaactttactcccttcctccccgctgaaagtactttacaacccgaaggccttcttcatacacgcngcatggctgcatcaggcttgcgcccattgtgcaatattccccactgctgcctcccgtaggagtctggaccgtgtctcagttccagtgttgctggtcatcctctcagaccagctagggatcgtcgcctaggtgagccgttaccccacctactagctaatcccatctgggcacatccgatggcaagaggccctaaggtccccctctttgtgcttgcgacgttatgcggtattagctaccgtttccagtagttatccccctccatcaggcagtttcccagacattactcacccgtccgccactcgtcagcaaagcagcaagctgcttcctgttaccgttcgacttgcatgtgttaggcctgccgccagcgttcaatctgagccatgatcaaact

SEQ ID NO: 25 - DNA, 1140 bp, Salmonella enterica
  subsp. enterica (T) ATCC 13311
  misc_feature 26: /note=" n= a or g or c or t/u"
taaggaggtgatccaaccgcaggttnccctacggttaccttgttacgacttcaccccagtcatgaatcacaaagtggtaagcgccctcccgaaggttaagctacctacttcttttgcaacccactcccatggtgtgacgggcggtgtgtacaaggcccgggaacgtattcaccgtggcattctgatccacgattactagcgattccgacttcatggagtcgagttgcagactccaatccggactacgacgcactttatgaggtccgcttgctctcgcgaggtcgcttctctttgtatgcgccattgtagcacgtgtgtagccctggtcgtaagggccatgatgacttgacgtcatccccaccttcctccagtttatcactggcagtctcctttgagttcccgacctaatcgctggcaacaaaggataagggttgcgctcgttgcgggacttaacccaacatttcacaacacgagctgacgacagccatgcagcacctgtctcacagttcccgaaggcaccaatccatctctggattcttctgtggatgtcaagaccaggtaaggttcttcgcgttgcatcgaattaaaccacatgctccaccgcttgtgcggcccccgtcaattcatttgagttttaaccttgcggccgtactccccaggcggtctacttaacgcgttacgtccggaagccacgcctcaagggcacaacctccaagtagacatcgtttacggcgtggactaccagggtatctaatcctgtttgctccccacgctttcgcacctgagcgtcagtctttgtccagggggccgccttcgccaccggtattcctccagatctctacgcatttcaccgctacacctggaattctacccccctctacaagactcaagcctgccagtttcgaatgcagttcccaggttgagcccggggatttcacatccgacttgacagaccgcctgcgtgcgctttacgcccagtaattccgattaacgcttgcaccctccgtattaccgcggctgctggcacggagttagccggtgcttcttctgcgggtaacgtcaattgctgcggttattaaccacaacaccttcctccccgctgaaagtactttacaacccgaaggccttcttcatacacgc

SEQ ID NO: 26 - DNA, 19 bp, Artificial Sequence
  RNase P Primer F
agatttggacctgcgagcg

SEQ ID NO: 27 - DNA, 20 bp, Artificial Sequence
  RNase P Primer R
gagcggctgtctccacaagt

SEQ ID NO: 28 - DNA, 23 bp, Artificial Sequence
  RNase P Probe
ttctgacctgaaggctctgcgcg

SEQ ID NO: 29 - DNA, 31 bp, Artificial Sequence
  RNase P Primer F with tag
gatcgatcgatcagatttggacctgcgagcg

SEQ ID NO: 30 - DNA, 12 bp, Artificial Sequence
  MiRNAX UNIVERAL Probe
gatcgatcgatc

SEQ ID NO: 31 - DNA, 12 bp, Artificial Sequence
  UNIVERAL Probe
gatcgatcgatc